European Patent Specification EP 3 823 665 B1, published January 24, 2024. Title: Chimeric Antigen Receptors with BCMA Specificity and Uses Thereof. Applicant: Regeneron Pharmaceuticals, Inc. The sequence listing filed with the application follows.

SEQUENCE LISTING (101 sequences)

SEQ ID NO: 1 - DNA, 366 bp, Artificial Sequence
  synthetic
caggtgcagctggtggagtcggggggaggcgtggtccagcctgggaggtccctgagactctcctgtgcagcctctggattcaccttcagtacctatggcattcactgggtccgccaggctccaggcaaggggctggagtgggtggcagttatattacatgatggaagtagtaactactatgcagagtccgtgaagggccgattcatcatctccagagacaattccaagaacacactgtatctgcaaatgaacagcctgagagctgaggacacggctctatattactgtacgaaaaggtattcagaagcagctggcccaaattggttcgacccctggggccagggaaccctggtcaccgtctcctca

SEQ ID NO: 2 - protein, 122 aa, Artificial Sequence
  synthetic
QVQLVESGGGVVQPGRSLRLSCAASGFTFSTYGIHWVRQAPGKGLEWVAVILHDGSSNYYAESVKGRFIISRDNSKNTLYLQMNSLRAEDTALYYCTKRYSEAAGPNWFDPWGQGTLVTVSS

SEQ ID NO: 3 - DNA, 24 bp, Artificial Sequence
  synthetic
ggattcaccttcagtacctatggc

SEQ ID NO: 4 - protein, 8 aa, Artificial Sequence
  synthetic
GFTFSTYG

SEQ ID NO: 5 - DNA, 24 bp, Artificial Sequence
  synthetic
atattacatgatggaagtagtaac

SEQ ID NO: 6 - protein, 8 aa, Artificial Sequence
  synthetic
ILHDGSSN

SEQ ID NO: 7 - DNA, 45 bp, Artificial Sequence
  synthetic
acgaaaaggtattcagaagcagctggcccaaattggttcgacccc

SEQ ID NO: 8 - protein, 15 aa, Artificial Sequence
  synthetic
TKRYSEAAGPNWFDP

SEQ ID NO: 9 - DNA, 321 bp, Artificial Sequence
  synthetic
gacatccagatgacccagtctccatcctccgtgtctgcatctgtaggagacagagtcaccatcacttgtcgggcgagtcggggaattagcagctggttagcctggtatcagcagaagccagggaaagcccctaagctcctgatccatgctgcatccagtttgcaaagtggggtcccatcaaggttcagcggcagtggatctgggacagatttcactctcaccatcagcagcctgcagcctgaagattttgctacttactattgtcaacaggctatcagtttcccattcactttcggccctgggaccaaagtggatatcaaa

SEQ ID NO: 10 - protein, 107 aa, Artificial Sequence
  synthetic
DIQMTQSPSSVSASVGDRVTITCRASRGISSWLAWYQQKPGKAPKLLIHAASSLQSGVPSRFSGSGSGTDFTLTISSLQPEDFATYYCQQAISFPFTFGPGTKVDIK

SEQ ID NO: 11 - DNA, 18 bp, Artificial Sequence
  synthetic
cggggaattagcagctgg

SEQ ID NO: 12 - protein, 6 aa, Artificial Sequence
  synthetic
RGISSW

SEQ ID NO: 13 - DNA, 9 bp, Artificial Sequence
  synthetic
gctgcatcc

SEQ ID NO: 14 - protein, 3 aa, Artificial Sequence
  synthetic
AAS

SEQ ID NO: 15 - DNA, 27 bp, Artificial Sequence
  synthetic
caacaggctatcagtttcccattcact

SEQ ID NO: 16 - protein, 9 aa, Artificial Sequence
  synthetic
QQAISFPFT

SEQ ID NO: 17 - DNA, 360 bp, Artificial Sequence
  synthetic
gaggtgcagctggtggagtctgggggaggcttggtacagcctggggggtccctgagactctcctgtgcagcctctggattcacctttagcagctatgtcatgagttgggtccgccaggctccagggaagggactggagtgggtctcagctattattggtagtggtggtagcacatattacgcagactccgtgaagggccggttcaccatctccagagacaattccaagaacacgctgtatctgcaaatgaacagcctgagagccgaggacacggccgtatattactgtgcgaaaagagccggggataactggaactggttcgacccctggggccagggaaccctggtcaccgtctcctca

SEQ ID NO: 18 - protein, 120 aa, Artificial Sequence
  synthetic
EVQLVESGGGLVQPGGSLRLSCAASGFTFSSYVMSWVRQAPGKGLEWVSAIIGSGGSTYYADSVKGRFTISRDNSKNTLYLQMNSLRAEDTAVYYCAKRAGDNWNWFDPWGQGTLVTVSS

SEQ ID NO: 19 - DNA, 24 bp, Artificial Sequence
  synthetic
ggattcacctttagcagctatgtc

SEQ ID NO: 20 - protein, 8 aa, Artificial Sequence
  synthetic
GFTFSSYV

SEQ ID NO: 21 - DNA, 24 bp, Artificial Sequence
  synthetic
attattggtagtggtggtagcaca

SEQ ID NO: 22 - protein, 8 aa, Artificial Sequence
  synthetic
IIGSGGST

SEQ ID NO: 23 - DNA, 39 bp, Artificial Sequence
  synthetic
gcgaaaagagccggggataactggaactggttcgacccc

SEQ ID NO: 24 - protein, 13 aa, Artificial Sequence
  synthetic
AKRAGDNWNWFDP

SEQ ID NO: 25 - DNA, 321 bp, Artificial Sequence
  synthetic
gacatccagatgacccagtctccatcttccgtgtctgcatctttaggagacagagtcaccatcacttgtcgggcgagtcagggtattagcagctggttagcctggtatcagcggaaaccagggaaagcccctaagctcctgatctatgctgcatccagtttgcaaagtggggtcccatcaaggttcagcggcagtggatctggggcggatttcactctcaccatcagcagcctgcagcctgaagattttgcaacttactattgtcaacaggctaaaagtgtcccattcactttcggccctgggaccaaagtggatatcaaa

SEQ ID NO: 26 - protein, 107 aa, Artificial Sequence
  synthetic
DIQMTQSPSSVSASLGDRVTITCRASQGISSWLAWYQRKPGKAPKLLIYAASSLQSGVPSRFSGSGSGADFTLTISSLQPEDFATYYCQQAKSVPFTFGPGTKVDIK

SEQ ID NO: 27 - DNA, 18 bp, Artificial Sequence
  synthetic
cagggtattagcagctgg

SEQ ID NO: 28 - protein, 6 aa, Artificial Sequence
  synthetic
QGISSW

SEQ ID NO: 29 - DNA, 9 bp, Artificial Sequence
  synthetic
gctgcatcc

SEQ ID NO: 30 - protein, 3 aa, Artificial Sequence
  synthetic
AAS

SEQ ID NO: 31 - DNA, 27 bp, Artificial Sequence
  synthetic
caacaggctaaaagtgtcccattcact

SEQ ID NO: 32 - protein, 9 aa, Artificial Sequence
  synthetic
QQAKSVPFT

SEQ ID NO: 33 - DNA, 351 bp, Artificial Sequence
  synthetic
gaagtgcagctggtggagtctgggggaggcttggtacagcctggcaggtccctgagactctcctgtgcagcctctggattcacctttgatgattatgccatgcactgggtccggcaagctccagggaagggcctggagtgggtctcaggtatcagttggaatagtggtaacatgggatatgcggactctgtgaagggccgattcaccatctccagagacaacgccaagaactccctgttcctgcaaatgcacagtttgagagctgaggacacggccttttattactgtgcaaaagtccgtctaactgcctttgacttttggggccagggaaccctggtcaccgtctcctca

SEQ ID NO: 34 - protein, 117 aa, Artificial Sequence
  synthetic
EVQLVESGGGLVQPGRSLRLSCAASGFTFDDYAMHWVRQAPGKGLEWVSGISWNSGNMGYADSVKGRFTISRDNAKNSLFLQMHSLRAEDTAFYYCAKVRLTAFDFWGQGTLVTVSS

SEQ ID NO: 35 - DNA, 24 bp, Artificial Sequence
  synthetic
ggattcacctttgatgattatgcc

SEQ ID NO: 36 - protein, 8 aa, Artificial Sequence
  synthetic
GFTFDDYA

SEQ ID NO: 37 - DNA, 24 bp, Artificial Sequence
  synthetic
atcagttggaatagtggtaacatg

SEQ ID NO: 38 - protein, 8 aa, Artificial Sequence
  synthetic
ISWNSGNM

SEQ ID NO: 39 - DNA, 30 bp, Artificial Sequence
  synthetic
gcaaaagtccgtctaactgcctttgacttt

SEQ ID NO: 40 - protein, 10 aa, Artificial Sequence
  synthetic
AKVRLTAFDF

SEQ ID NO: 41 - DNA, 321 bp, Artificial Sequence
  synthetic
gacatccagatgacccagtctccatcctccctgtctgcatctgtaggagacagagtcaccatcacttgccggacaagtcagagcattggcaactatttaaattggtttcagcagaaaccagggaaagcccctaaactcctcatctatactgcatccagtttgcagaatggagtcccatcaaggttcactggcagtggatctgggacagatttcactctcaccatcagcagtctgcaacctgaggattttgtaatttactactgtcaacagagtttcagtaccccgtatacttttggccaggggaccaagctggagatcaaa

SEQ ID NO: 42 - protein, 107 aa, Artificial Sequence
  synthetic
DIQMTQSPSSLSASVGDRVTITCRTSQSIGNYLNWFQQKPGKAPKLLIYTASSLQNGVPSRFTGSGSGTDFTLTISSLQPEDFVIYYCQQSFSTPYTFGQGTKLEIK

SEQ ID NO: 43 - DNA, 18 bp, Artificial Sequence
  synthetic
cagagcattggcaactat

SEQ ID NO: 44 - protein, 6 aa, Artificial Sequence
  synthetic
QSIGNY

SEQ ID NO: 45 - DNA, 9 bp, Artificial Sequence
  synthetic
actgcatcc

SEQ ID NO: 46 - protein, 3 aa, Artificial Sequence
  synthetic
TAS

SEQ ID NO: 47 - DNA, 27 bp, Artificial Sequence
  synthetic
caacagagtttcagtaccccgtatact

SEQ ID NO: 48 - protein, 9 aa, Artificial Sequence
  synthetic
QQSFSTPYT

SEQ ID NO: 49 - DNA, 354 bp, Artificial Sequence
  synthetic
caggtgcagctggtggagtctgggggaggcttggtcaagcctggagggtccctgagactctcctgtgcagcctctggattcaccttcagtgactactacatcagctggatccgccaggctccagggaaggggctggagtgggtttcatacattagttctagtggtagttccataaagtacgcagactctgtgaagggccgattcaccatctccagggacaacgccaagaactcactgtatctgcaaatgaacagcctgagagccgaggacacggccgtatattactgtgcgagagagggagggaactacggtatggacgtctggggccaagggaccacggtcaccgtctcctca

SEQ ID NO: 50 - protein, 118 aa, Artificial Sequence
  synthetic
QVQLVESGGGLVKPGGSLRLSCAASGFTFSDYYISWIRQAPGKGLEWVSYISSSGSSIKYADSVKGRFTISRDNAKNSLYLQMNSLRAEDTAVYYCAREGGNYGMDVWGQGTTVTVSS

SEQ ID NO: 51 - DNA, 24 bp, Artificial Sequence
  synthetic
ggattcaccttcagtgactactac

SEQ ID NO: 52 - protein, 8 aa, Artificial Sequence
  synthetic
GFTFSDYY

SEQ ID NO: 53 - DNA, 24 bp, Artificial Sequence
  synthetic
attagttctagtggtagttccata

SEQ ID NO: 54 - protein, 8 aa, Artificial Sequence
  synthetic
ISSSGSSI

SEQ ID NO: 55 - DNA, 33 bp, Artificial Sequence
  synthetic
gcgagagagggagggaactacggtatggacgtc

SEQ ID NO: 56 - protein, 11 aa, Artificial Sequence
  synthetic
AREGGNYGMDV

SEQ ID NO: 57 - DNA, 321 bp, Artificial Sequence
  synthetic
gacatccagatgacccagtctccatcttccgtgtctgcatctgtaggagacagagtcaccatcacttgtcgggcgagtcagggtattaacaactggttagtctggtatcagcagaaaccagggaaagcccctaagctcctgatctatgctgcaaccagcttgcaaagtggggtcccatcaaggttcagcggcagtgggtctgggacagatttcactctcaccatcagcagcctgcagcctgaagattttgcaacttactattgtcaacaggctaacagtttccctcccacttttggccaggggaccaagctggagatcaaa

SEQ ID NO: 58 - protein, 107 aa, Artificial Sequence
  synthetic
DIQMTQSPSSVSASVGDRVTITCRASQGINNWLVWYQQKPGKAPKLLIYAATSLQSGVPSRFSGSGSGTDFTLTISSLQPEDFATYYCQQANSFPPTFGQGTKLEIK

SEQ ID NO: 59 - DNA, 18 bp, Artificial Sequence
  synthetic
cagggtattaacaactgg

SEQ ID NO: 60 - protein, 6 aa, Artificial Sequence
  synthetic
QGINNW

SEQ ID NO: 61 - DNA, 9 bp, Artificial Sequence
  synthetic
gctgcaacc

SEQ ID NO: 62 - protein, 3 aa, Artificial Sequence
  synthetic
AAT

SEQ ID NO: 63 - DNA, 27 bp, Artificial Sequence
  synthetic
caacaggctaacagtttccctcccact

SEQ ID NO: 64 - protein, 9 aa, Artificial Sequence
  synthetic
QQANSFPPT

SEQ ID NO: 65 - DNA, 375 bp, Artificial Sequence
  synthetic
gaggtgcagctggtggagtctgggggaggcttggtccagcctggggggtccctgagactctcctgtgcagcctctggattcacctttagtaacttttggatgacctgggtccgccaggctccagggaaggggctggagtgggtggccaacatgaaccaagatggaagtgagaaatactatgtggactctgtgaagggccgattcaccatctccagagacaacgccaagagctcactgtatctgcaaatgaacagcctgagagccgaggacacggctgtgtattactgtgcgagagatcgggaatattgtattagtaccagctgctatgatgactttgactactggggccagggaaccctggtcaccgtctcctca

SEQ ID NO: 66 - protein, 125 aa, Artificial Sequence
  synthetic
EVQLVESGGGLVQPGGSLRLSCAASGFTFSNFWMTWVRQAPGKGLEWVANMNQDGSEKYYVDSVKGRFTISRDNAKSSLYLQMNSLRAEDTAVYYCARDREYCISTSCYDDFDYWGQGTLVTVSS

SEQ ID NO: 67 - DNA, 24 bp, Artificial Sequence
  synthetic
ggattcacctttagtaacttttgg

SEQ ID NO: 68 - protein, 8 aa, Artificial Sequence
  synthetic
GFTFSNFW

SEQ ID NO: 69 - DNA, 24 bp, Artificial Sequence
  synthetic
atgaaccaagatggaagtgagaaa

SEQ ID NO: 70 - protein, 8 aa, Artificial Sequence
  synthetic
MNQDGSEK

SEQ ID NO: 71 - DNA, 54 bp, Artificial Sequence
  synthetic
gcgagagatcgggaatattgtattagtaccagctgctatgatgactttgactac

SEQ ID NO: 72 - protein, 18 aa, Artificial Sequence
  synthetic
ARDREYCISTSCYDDFDY

SEQ ID NO: 73 - DNA, 324 bp, Artificial Sequence
  synthetic
gacatccagatgacccagtctccatcctccctgtctgcatctgtaggagacagagtcaccatcacttgccgggcaagtcagagcattagcagctatttaaattggtatcagcagaaaccagggaaagcccctaagctcctgatctatgctgcatccagtttgcatagtggggtcccatcaaggttcagtggcagtggatctgggacagatttcactctcaccatcagcagtctgcaacctgaagattttgcaacttactactgtcaacagagttacagtacccctccgatcaccttcggccaagggacacgactggagattaaa

SEQ ID NO: 74 - protein, 108 aa, Artificial Sequence
  synthetic
DIQMTQSPSSLSASVGDRVTITCRASQSISSYLNWYQQKPGKAPKLLIYAASSLHSGVPSRFSGSGSGTDFTLTISSLQPEDFATYYCQQSYSTPPITFGQGTRLEIK

SEQ ID NO: 75 - DNA, 18 bp, Artificial Sequence
  synthetic
cagagcattagcagctat

SEQ ID NO: 76 - protein, 6 aa, Artificial Sequence
  synthetic
QSISSY

SEQ ID NO: 77 - DNA, 9 bp, Artificial Sequence
  synthetic
gctgcatcc

SEQ ID NO: 78 - protein, 3 aa, Artificial Sequence
  synthetic
AAS

SEQ ID NO: 79 - DNA, 30 bp, Artificial Sequence
  synthetic
caacagagttacagtacccctccgatcacc

SEQ ID NO: 80 - protein, 10 aa, Artificial Sequence
  synthetic
QQSYSTPPIT

SEQ ID NO: 81 - DNA, 1404 bp, Artificial Sequence
  BCMA 16711 (VL-VH) ScFv CAR-T (16711_VK_v2(human).(G4S)3 Linker.16711 VH.hCD8a hinge/TM.hCD137 (4-1BB).hCD3 zeta)
gacatccagatgacccagtctccatcctccgtgtctgcatctgtaggagacagagtcaccatcacttgtcgggcgagtcggggaattagcagctggttagcctggtatcagcagaagccagggaaagcccctaagctcctgatccatgctgcatccagtttgcaaagtggggtcccatcaaggttcagcggcagtggatctgggacagatttcactctcaccatcagcagcctgcagcctgaagattttgctacttactattgtcaacaggctatcagtttcccattcactttcggccctgggaccaaagtggatatcaaaggcggcggtggatctggaggcggtggaagcggtggcgggggaagtcaggtgcagctggtggagtcggggggaggcgtggtccagcctgggaggtccctgagactctcctgtgcagcctctggattcaccttcagtacctatggcattcactgggtccgccaggctccaggcaaggggctggagtgggtggcagttatattacatgatggaagtagtaactactatgcagagtccgtgaagggccgattcatcatctccagagacaattccaagaacacactgtatctgcaaatgaacagcctgagagctgaggacacggctctatattactgtacgaaaaggtattcagaagcagctggcccaaattggttcgacccctggggccagggaaccctggtcaccgtctcctcaactaccactcctgctccccgccccccaacacctgctccaactattgcatcccaaccactctccctcagacccgaagcttgtcgccccgccgccggaggtgctgttcacactagaggactcgattttgcttgcgacatttatatctgggccccacttgcaggtacttgcggagtattgctgctctcacttgttattactctttattgcaaacggggcagaaagaaactcctgtatatattcaaacaaccatttatgagaccagtacaaactactcaagaggaagatggctgtagctgccgatttccagaagaagaagaaggaggatgtgaactgagagtgaagttcagcaggagcgcagacgcccccgcgtacaagcagggccagaaccagctctataacgagctcaatctaggacgaagagaggagtacgatgttttggacaagagacgtggccgggaccctgagatggggggaaagccgagaaggaagaaccctcaggaaggcctgtacaatgaactgcagaaagataagatggcggaggcctacagtgagattgggatgaaaggcgagcgccggaggggcaaggggcacgatggcctttaccagggtctcagtacagccaccaaggacacctacgacgcccttcacatgcaggccctgccccctcgctaa

SEQ ID NO: 82 - protein, 467 aa, Artificial Sequence
  BCMA 16711 (VL-VH) ScFv CAR-T (16711_VK_v2(human).(G4S)3 Linker.16711 VH.hCD8a hinge/TM.hCD137 (4-1BB).hCD3 zeta)
DIQMTQSPSSVSASVGDRVTITCRASRGISSWLAWYQQKPGKAPKLLIHAASSLQSGVPSRFSGSGSGTDFTLTISSLQPEDFATYYCQQAISFPFTFGPGTKVDIKGGGGSGGGGSGGGGSQVQLVESGGGVVQPGRSLRLSCAASGFTFSTYGIHWVRQAPGKGLEWVAVILHDGSSNYYAESVKGRFIISRDNSKNTLYLQMNSLRAEDTALYYCTKRYSEAAGPNWFDPWGQGTLVTVSSTTTPAPRPPTPAPTIASQPLSLRPEACRPAAGGAVHTRGLDFACDIYIWAPLAGTCGVLLLSLVITLYCKRGRKKLLYIFKQPFMRPVQTTQEEDGCSCRFPEEEEGGCELRVKFSRSADAPAYKQGQNQLYNELNLGRREEYDVLDKRRGRDPEMGGKPRRKNPQEGLYNELQKDKMAEAYSEIGMKGERRRGKGHDGLYQGLSTATKDTYDALHMQALPPR

SEQ ID NO: 83 - DNA, 1398 bp, Artificial Sequence
  BCMA 16716 (VL-VH) ScFv CAR-T (16716_VK(human).(G4S)3 Linker.16716_VH(human).hCD8a hinge/TM.hCD137 (4-1BB).hCD3 zeta)
gacatccagatgacccagtctccatcttccgtgtctgcatctttaggagacagagtcaccatcacttgtcgggcgagtcagggtattagcagctggttagcctggtatcagcggaaaccagggaaagcccctaagctcctgatctatgctgcatccagtttgcaaagtggggtcccatcaaggttcagcggcagtggatctggggcggatttcactctcaccatcagcagcctgcagcctgaagattttgcaacttactattgtcaacaggctaaaagtgtcccattcactttcggccctgggaccaaagtggatatcaaaggcggcggtggatctggaggcggtggaagcggtggcgggggaagtgaggtgcagctggtggagtctgggggaggcttggtacagcctggggggtccctgagactctcctgtgcagcctctggattcacctttagcagctatgtcatgagttgggtccgccaggctccagggaagggactggagtgggtctcagctattattggtagtggtggtagcacatattacgcagactccgtgaagggccggttcaccatctccagagacaattccaagaacacgctgtatctgcaaatgaacagcctgagagccgaggacacggccgtatattactgtgcgaaaagagccggggataactggaactggttcgacccctggggccagggaaccctggtcaccgtctcctcaactaccactcctgctccccgccccccaacacctgctccaactattgcatcccaaccactctccctcagacccgaagcttgtcgccccgccgccggaggtgctgttcacactagaggactcgattttgcttgcgacatttatatctgggccccacttgcaggtacttgcggagtattgctgctctcacttgttattactctttattgcaaacggggcagaaagaaactcctgtatatattcaaacaaccatttatgagaccagtacaaactactcaagaggaagatggctgtagctgccgatttccagaagaagaagaaggaggatgtgaactgagagtgaagttcagcaggagcgcagacgcccccgcgtacaagcagggccagaaccagctctataacgagctcaatctaggacgaagagaggagtacgatgttttggacaagagacgtggccgggaccctgagatggggggaaagccgagaaggaagaaccctcaggaaggcctgtacaatgaactgcagaaagataagatggcggaggcctacagtgagattgggatgaaaggcgagcgccggaggggcaaggggcacgatggcctttaccagggtctcagtacagccaccaaggacacctacgacgcccttcacatgcaggccctgccccctcgctaa

SEQ ID NO: 84 - protein, 465 aa, Artificial Sequence
  BCMA 16716 (VL-VH) ScFv CAR-T (16716_VK(human).(G4S)3 Linker.16716_VH(human).hCD8a hinge/TM.hCD137 (4-1BB).hCD3 zeta)
DIQMTQSPSSVSASLGDRVTITCRASQGISSWLAWYQRKPGKAPKLLIYAASSLQSGVPSRFSGSGSGADFTLTISSLQPEDFATYYCQQAKSVPFTFGPGTKVDIKGGGGSGGGGSGGGGSEVQLVESGGGLVQPGGSLRLSCAASGFTFSSYVMSWVRQAPGKGLEWVSAIIGSGGSTYYADSVKGRFTISRDNSKNTLYLQMNSLRAEDTAVYYCAKRAGDNWNWFDPWGQGTLVTVSSTTTPAPRPPTPAPTIASQPLSLRPEACRPAAGGAVHTRGLDFACDIYIWAPLAGTCGVLLLSLVITLYCKRGRKKLLYIFKQPFMRPVQTTQEEDGCSCRFPEEEEGGCELRVKFSRSADAPAYKQGQNQLYNELNLGRREEYDVLDKRRGRDPEMGGKPRRKNPQEGLYNELQKDKMAEAYSEIGMKGERRRGKGHDGLYQGLSTATKDTYDALHMQALPPR

SEQ ID NO: 85 - DNA, 1389 bp, Artificial Sequence
  BCMA 16732 (VL-VH) ScFv CAR-T (16732_VK_v2(human).(G4S)3 Linker.16732_VH(human).hCD8a hinge/TM.hCD137 (4-1BB).hCD3 zeta)
gacatccagatgacccagtctccatcctccctgtctgcatctgtaggagacagagtcaccatcacttgccggacaagtcagagcattggcaactatttaaattggtttcagcagaaaccagggaaagcccctaaactcctcatctatactgcatccagtttgcagaatggagtcccatcaaggttcactggcagtggatctgggacagatttcactctcaccatcagcagtctgcaacctgaggattttgtaatttactactgtcaacagagtttcagtaccccgtatacttttggccaggggaccaagctggagatcaaaggcggcggtggatctggaggcggtggaagcggtggcgggggaagtgaagtgcagctggtggagtctgggggaggcttggtacagcctggcaggtccctgagactctcctgtgcagcctctggattcacctttgatgattatgccatgcactgggtccggcaagctccagggaagggcctggagtgggtctcaggtatcagttggaatagtggtaacatgggatatgcggactctgtgaagggccgattcaccatctccagagacaacgccaagaactccctgttcctgcaaatgcacagtttgagagctgaggacacggccttttattactgtgcaaaagtccgtctaactgcctttgacttttggggccagggaaccctggtcaccgtctcctcaactaccactcctgctccccgccccccaacacctgctccaactattgcatcccaaccactctccctcagacccgaagcttgtcgccccgccgccggaggtgctgttcacactagaggactcgattttgcttgcgacatttatatctgggccccacttgcaggtacttgcggagtattgctgctctcacttgttattactctttattgcaaacggggcagaaagaaactcctgtatatattcaaacaaccatttatgagaccagtacaaactactcaagaggaagatggctgtagctgccgatttccagaagaagaagaaggaggatgtgaactgagagtgaagttcagcaggagcgcagacgcccccgcgtacaagcagggccagaaccagctctataacgagctcaatctaggacgaagagaggagtacgatgttttggacaagagacgtggccgggaccctgagatggggggaaagccgagaaggaagaaccctcaggaaggcctgtacaatgaactgcagaaagataagatggcggaggcctacagtgagattgggatgaaaggcgagcgccggaggggcaaggggcacgatggcctttaccagggtctcagtacagccaccaaggacacctacgacgcccttcacatgcaggccctgccccctcgctaa

SEQ ID NO: 86 - protein, 462 aa, Artificial Sequence
  BCMA 16732 (VL-VH) ScFv CAR-T (16732_VK_v2(human).(G4S)3 Linker.16732_VH(human).hCD8a hinge/TM.hCD137 (4-1BB).hCD3 zeta)
DIQMTQSPSSLSASVGDRVTITCRTSQSIGNYLNWFQQKPGKAPKLLIYTASSLQNGVPSRFTGSGSGTDFTLTISSLQPEDFVIYYCQQSFSTPYTFGQGTKLEIKGGGGSGGGGSGGGGSEVQLVESGGGLVQPGRSLRLSCAASGFTFDDYAMHWVRQAPGKGLEWVSGISWNSGNMGYADSVKGRFTISRDNAKNSLFLQMHSLRAEDTAFYYCAKVRLTAFDFWGQGTLVTVSSTTTPAPRPPTPAPTIASQPLSLRPEACRPAAGGAVHTRGLDFACDIYIWAPLAGTCGVLLLSLVITLYCKRGRKKLLYIFKQPFMRPVQTTQEEDGCSCRFPEEEEGGCELRVKFSRSADAPAYKQGQNQLYNELNLGRREEYDVLDKRRGRDPEMGGKPRRKNPQEGLYNELQKDKMAEAYSEIGMKGERRRGKGHDGLYQGLSTATKDTYDALHMQALPPR

SEQ ID NO: 87 - DNA, 1392 bp, Artificial Sequence
  BCMA 16747 (VL-VH) ScFv CAR-T (16747_VK(human).(G4S)3 Linker.16747_VH(human).hCD8a hinge/TM.hCD137 (4-1BB).hCD3 zeta)
gacatccagatgacccagtctccatcttccgtgtctgcatctgtaggagacagagtcaccatcacttgtcgggcgagtcagggtattaacaactggttagtctggtatcagcagaaaccagggaaagcccctaagctcctgatctatgctgcaaccagcttgcaaagtggggtcccatcaaggttcagcggcagtgggtctgggacagatttcactctcaccatcagcagcctgcagcctgaagattttgcaacttactattgtcaacaggctaacagtttccctcccacttttggccaggggaccaagctggagatcaaaggcggcggtggatctggaggcggtggaagcggtggcgggggaagtcaggtgcagctggtggagtctgggggaggcttggtcaagcctggagggtccctgagactctcctgtgcagcctctggattcaccttcagtgactactacatcagctggatccgccaggctccagggaaggggctggagtgggtttcatacattagttctagtggtagttccataaagtacgcagactctgtgaagggccgattcaccatctccagggacaacgccaagaactcactgtatctgcaaatgaacagcctgagagccgaggacacggccgtatattactgtgcgagagagggagggaactacggtatggacgtctggggccaagggaccacggtcaccgtctcctcaactaccactcctgctccccgccccccaacacctgctccaactattgcatcccaaccactctccctcagacccgaagcttgtcgccccgccgccggaggtgctgttcacactagaggactcgattttgcttgcgacatttatatctgggccccacttgcaggtacttgcggagtattgctgctctcacttgttattactctttattgcaaacggggcagaaagaaactcctgtatatattcaaacaaccatttatgagaccagtacaaactactcaagaggaagatggctgtagctgccgatttccagaagaagaagaaggaggatgtgaactgagagtgaagttcagcaggagcgcagacgcccccgcgtacaagcagggccagaaccagctctataacgagctcaatctaggacgaagagaggagtacgatgttttggacaagagacgtggccgggaccctgagatggggggaaagccgagaaggaagaaccctcaggaaggcctgtacaatgaactgcagaaagataagatggcggaggcctacagtgagattgggatgaaaggcgagcgccggaggggcaaggggcacgatggcctttaccagggtctcagtacagccaccaaggacacctacgacgcccttcacatgcaggccctgccccctcgctaa

SEQ ID NO: 88 - protein, 463 aa, Artificial Sequence
  BCMA 16747 (VL-VH) ScFv CAR-T (16747_VK(human).(G4S)3 Linker.16747_VH(human).hCD8a hinge/TM.hCD137 (4-1BB).hCD3 zeta)
DIQMTQSPSSVSASVGDRVTITCRASQGINNWLVWYQQKPGKAPKLLIYAATSLQSGVPSRFSGSGSGTDFTLTISSLQPEDFATYYCQQANSFPPTFGQGTKLEIKGGGGSGGGGSGGGGSQVQLVESGGGLVKPGGSLRLSCAASGFTFSDYYISWIRQAPGKGLEWVSYISSSGSSIKYADSVKGRFTISRDNAKNSLYLQMNSLRAEDTAVYYCAREGGNYGMDVWGQGTTVTVSSTTTPAPRPPTPAPTIASQPLSLRPEACRPAAGGAVHTRGLDFACDIYIWAPLAGTCGVLLLSLVITLYCKRGRKKLLYIFKQPFMRPVQTTQEEDGCSCRFPEEEEGGCELRVKFSRSADAPAYKQGQNQLYNELNLGRREEYDVLDKRRGRDPEMGGKPRRKNPQEGLYNELQKDKMAEAYSEIGMKGERRRGKGHDGLYQGLSTATKDTYDALHMQALPPR

SEQ ID NO: 89 - DNA, 1431 bp, Artificial Sequence
  BCMA 21581 (VL-VH) ScFv CAR-T (21581 VK(human).(G4S)3 Linker.21581 VH(human).G4S Linker_v2.hCD8a hinge/TM.hCD137 (4-1BB).hCD3 zeta)
gacatccagatgacccagtctccatcctccctgtctgcatctgtaggagacagagtcaccatcacttgccgggcaagtcagagcattagcagctatttaaattggtatcagcagaaaccagggaaagcccctaagctcctgatctatgctgcatccagtttgcatagtggggtcccatcaaggttcagtggcagtggatctgggacagatttcactctcaccatcagcagtctgcaacctgaagattttgcaacttactactgtcaacagagttacagtacccctccgatcaccttcggccaagggacacgactggagattaaaggcggcggtggatctggaggcggtggaagcggtggcgggggaagtgaggtgcagctggtggagtctgggggaggcttggtccagcctggggggtccctgagactctcctgtgcagcctctggattcacctttagtaacttttggatgacctgggtccgccaggctccagggaaggggctggagtgggtggccaacatgaaccaagatggaagtgagaaatactatgtggactctgtgaagggccgattcaccatctccagagacaacgccaagagctcactgtatctgcaaatgaacagcctgagagccgaggacacggctgtgtattactgtgcgagagatcgggaatattgtattagtaccagctgctatgatgactttgactactggggccagggaaccctggtcaccgtctcctcaggaggcggaggcagcactaccactcctgctccccgccccccaacacctgctccaactattgcatcccaaccactctccctcagacccgaagcttgtcgccccgccgccggaggtgctgttcacactagaggactcgattttgcttgcgacatttatatctgggccccacttgcaggtacttgcggagtattgctgctctcacttgttattactctttattgcaaacggggcagaaagaaactcctgtatatattcaaacaaccatttatgagaccagtacaaactactcaagaggaagatggctgtagctgccgatttccagaagaagaagaaggaggatgtgaactgagagtgaagttcagcaggagcgcagacgcccccgcgtacaagcagggccagaaccagctctataacgagctcaatctaggacgaagagaggagtacgatgttttggacaagagacgtggccgggaccctgagatggggggaaagccgagaaggaagaaccctcaggaaggcctgtacaatgaactgcagaaagataagatggcggaggcctacagtgagattgggatgaaaggcgagcgccggaggggcaaggggcacgatggcctttaccagggtctcagtacagccaccaaggacacctacgacgcccttcacatgcaggccctgccccctcgctaa

SEQ ID NO: 90 - protein, 476 aa, Artificial Sequence
  BCMA 21581 (VL-VH) ScFv CAR-T (21581 VK(human).(G4S)3 Linker.21581 VH(human).G4S Linker_v2.hCD8a hinge/TM.hCD137 (4-1BB).hCD3 zeta)
DIQMTQSPSSLSASVGDRVTITCRASQSISSYLNWYQQKPGKAPKLLIYAASSLHSGVPSRFSGSGSGTDFTLTISSLQPEDFATYYCQQSYSTPPITFGQGTRLEIKGGGGSGGGGSGGGGSEVQLVESGGGLVQPGGSLRLSCAASGFTFSNFWMTWVRQAPGKGLEWVANMNQDGSEKYYVDSVKGRFTISRDNAKSSLYLQMNSLRAEDTAVYYCARDREYCISTSCYDDFDYWGQGTLVTVSSGGGGSTTTPAPRPPTPAPTIASQPLSLRPEACRPAAGGAVHTRGLDFACDIYIWAPLAGTCGVLLLSLVITLYCKRGRKKLLYIFKQPFMRPVQTTQEEDGCSCRFPEEEEGGCELRVKFSRSADAPAYKQGQNQLYNELNLGRREEYDVLDKRRGRDPEMGGKPRRKNPQEGLYNELQKDKMAEAYSEIGMKGERRRGKGHDGLYQGLSTATKDTYDALHMQALPPR

SEQ ID NO: 91 - DNA, 1437 bp, Artificial Sequence
  HLA-A2/HPV16E7(11-19) 17363 ScFv (VL-VH) CAR-T (Irrelevant Control) (17363_ULC-VK(1)(human).G4Sx3_4.17363_VH(human). G4S_V2.hCD8a hinge/TM.hCD137 (4-1BB).hCD3 zeta)
gacatccagatgacccagtctccatcctccctgtctgcatctgtaggagacagagtcaccatcacttgccgggcaagtcagagcattagcagctatttaaattggtatcaacagaaaccagggaaagcccctaagctcctgatctatgctgtttccattttgcaaagtggggtcccatcaaggttcagtggcagtggatctgggacagatttcactctcaccatcaactctctgcaacctgaagattttgcaacttactcctgtcaacagacttacagtacccctccgatcaccttcggccaagggacacgactggagattaaaggtggaggcggtagtggcggaggcggaagtggtggaggaggctcagaggtgcagctgttggagtctgggggaggcttggtacaacctggggggtccctgagactctcctgtgcagcctctggattcacctttagcagttatgccatgacctgggtccgccaggctccagggatgggactggagtgggtctcagttattagtggtagtggtagtgaaacatactacgcagactccgtgaagggccggttcaccatctccagagacaattccaaaaacacactgtatctgcaaatgaacagcctgagagccgaagacacggccgtatattactgtgtgaaagattcttcgtataggagctcgtcgagggcctactactactacggaatggacgtctggggcctagggaccacggtcaccgtctcctcaggaggtggtggaagtactaccactcctgctccccgccccccaacacctgctccaactattgcatcccaaccactctccctcagacccgaagcttgtcgccccgccgccggaggtgctgttcacactagaggactcgattttgcttgcgacatttatatctgggccccacttgcaggtacttgcggagtattgctgctctcacttgttattactctttattgcaaacggggcagaaagaaactcctgtatatattcaaacaaccatttatgagaccagtacaaactactcaagaggaagatggctgtagctgccgatttccagaagaagaagaaggaggatgtgaactgagagtgaagttcagcaggagcgcagacgcccccgcgtacaagcagggccagaaccagctctataacgagctcaatctaggacgaagagaggagtacgatgttttggacaagagacgtggccgggaccctgagatggggggaaagccgagaaggaagaaccctcaggaaggcctgtacaatgaactgcagaaagataagatggcggaggcctacagtgagattgggatgaaaggcgagcgccggaggggcaaggggcacgatggcctttaccagggtctcagtacagccaccaaggacacctacgacgcccttcacatgcaggccctgccccctcgctaa

SEQ ID NO: 92 - protein, 478 aa, Artificial Sequence
  HLA-A2/HPV16E7(11-19) 17363 ScFv (VL-VH) CAR-T (Irrelevant Control) (17363_ULC-VK(1)(human).G4Sx3_4.17363_VH(human). G4S_V2.hCD8a hinge/TM.hCD137 (4-1BB).hCD3 zeta)
DIQMTQSPSSLSASVGDRVTITCRASQSISSYLNWYQQKPGKAPKLLIYAVSILQSGVPSRFSGSGSGTDFTLTINSLQPEDFATYSCQQTYSTPPITFGQGTRLEIKGGGGSGGGGSGGGGSEVQLLESGGGLVQPGGSLRLSCAASGFTFSSYAMTWVRQAPGMGLEWVSVISGSGSETYYADSVKGRFTISRDNSKNTLYLQMNSLRAEDTAVYYCVKDSSYRSSSRAYYYYGMDVWGLGTTVTVSSGGGGSTTTPAPRPPTPAPTIASQPLSLRPEACRPAAGGAVHTRGLDFACDIYIWAPLAGTCGVLLLSLVITLYCKRGRKKLLYIFKQPFMRPVQTTQEEDGCSCRFPEEEEGGCELRVKFSRSADAPAYKQGQNQLYNELNLGRREEYDVLDKRRGRDPEMGGKPRRKNPQEGLYNELQKDKMAEAYSEIGMKGERRRGKGHDGLYQGLSTATKDTYDALHMQALPPR

SEQ ID NO: 93 - protein, 5 aa, Artificial Sequence
  linker
GGGGS

SEQ ID NO: 94 - protein, 10 aa, Artificial Sequence
  linker
GGGGSGGGGS

SEQ ID NO: 95 - protein, 15 aa, Artificial Sequence
  linker
GGGGSGGGGSGGGGS

SEQ ID NO: 96 - protein, 18 aa, Artificial Sequence
  linker
GSTSGSGKPGSGEGSTKG

SEQ ID NO: 97 - protein, 45 aa, Artificial Sequence
  hinge
TTTPAPRPPTPAPTIASQPLSLRPEACRPAAGGAVHTRGLDFACD

SEQ ID NO: 98 - protein, 24 aa, Artificial Sequence
  TM domain
IYIWAPLAGTCGVLLLSLVITLYC

SEQ ID NO: 99 - protein, 42 aa, Artificial Sequence
  4-1BB
KRGRKKLLYIFKQPFMRPVQTTQEEDGCSCRFPEEEEGGCEL

SEQ ID NO: 100 - protein, 112 aa, Artificial Sequence
  cd3-Zeta
RVKFSRSADAPAYKQGQNQLYNELNLGRREEYDVLDKRRGRDPEMGGKPRRKNPQEGLYNELQKDKMAEAYSEIGMKGERRRGKGHDGLYQGLSTATKDTYDALHMQALPPR

SEQ ID NO: 101 - protein, 184 aa, Artificial Sequence
  human BCMA (TNFRSF17) Protein NP_001183.2
MLQMAGQCSQNEYFDSLLHACIPCQLRCSSNTPPLTCQRYCNASVTNSVKGTNAILWTCLGLSLIISLAVFVLMFLLRKINSEPLKDEFKNTGSGLLGMANIDLEKSRTGDEIILPRGLEYTVEECTCEDCIKSKPKVDSDHCFPLPAMEEGATILVTTKTNDYCKSLPAALSATEIEKSISAR